European Patent Specification EP 3 517 542 B1, published October 25, 2023. Title: Dendric cell targetting peptide, fusion petide containing the same, and vacine using the fusion peptide. Applicant: The Research Foundation for Microbial Diseases of Osaka University. The sequence listing filed with the application follows.

SEQUENCE LISTING (6 sequences)

SEQ ID NO: 1 - protein, 7 aa, Artificial Sequence
  Amino acid sequence of motif sequence
VSYKAIR

SEQ ID NO: 2 - protein, 7 aa, Artificial Sequence
  Amino acid sequence of motif sequence
ASYKAIR

SEQ ID NO: 3 - protein, 7 aa, Artificial Sequence
  Amino acid sequence of motif sequence
VAYKAIR

SEQ ID NO: 4 - DNA, 21 bp, Artificial Sequence
  Base sequence of a peptide having a motif sequence
gtgagctataaagcgattcgt

SEQ ID NO: 5 - DNA, 63 bp, Artificial Sequence
  Base sequence of a peptide having three motif sequences
gtgagctataaagcgattcgtgtgagctataaagcgattcgtgtgagctataaagcgattcgt

SEQ ID NO: 6 - DNA, 1140 bp, Pneumococcus
atggaagaatctcccgtagctagtcagtctaaagctgagaaagactatgatgcagcagtgaaaaaatctgaagctgctaagaaggcttacgaagaagctaaaaaagctttagaggaagcaaaagttgcgcaaaaaaaatatgaagacgatcaaaagaaaactgaagagaaagcagagctagaaaaagaagcttctgaagcgatagctaaggcaacagaagaagttcaacaagcgtacctagcttatcaacgagctagcaacaaagccgaagcagctaagatgatagaagaggctcagagacgcgaaaatgaggcgagagctaaatttactactattcgaacaacaatggtagttcctgaaccagaacagttagctgagactaagaaaaaagcagaagaagctaaagcaaaagaaccaaaacttgctaaaaaagcagcagaagctaaagcaaaattagaagaggctgagaaaaaagctactgaagccaaacaaaaagtggatgctgaagaagtcgctcctcaagctaaaatcgctgaattggaaaatcaagttcatagactagaacaagagctcaaagagattgatgagtctgaatcagaagattatgctaaagaaggtttccgtgctcctcttcaatctaaattggatgccaaaaaagctaaactatcaaaacttgaagagttaagtgataagattgatgagttagacgctgaaattgcaaaacttgaagatcaacttaaagctgctgaagaaaacaataatgtagaagactactttaaagaaggtttagagaaaactattgctgctaaaaaagctgaattagaaaaaactgaagctgaccttaagaaagcagttaatgagccagaaaaatcagctgaagagccatcgcaaccagagaagccagctgaagaagctccagccccagagcaaccaactgagccaactcaaccagaaaaaccagctgaagaaactccagcaccaaaaccagagaagccagctgaacaaccaaaagcagaaaaaacagatgatcaacaagctgaagaagactatgctcgtagatcagaagaagaatataatcgcttgactcaacagcaaccgccaaaagcagaaaaaccagctcctgcaccacaaccagagtaa